European Patent Specification EP 4 136 092 B1, published July 31, 2024. Title: COMPOUNDS AND METHODS FOR MODULATING ANGIOTENSINOGEN EXPRESSION. Applicant: Ionis Pharmaceuticals, Inc. The sequence listing filed with the application follows.

SEQUENCE LISTING (28 sequences)

SEQ ID NO: 1 - DNA, 2587 bp, Homo sapiens
atcccatgagcgggcagcagggtcagaagtggcccccgtgttgcctaagcaagactctcccctgccctctgccctctgcacctccggcctgcatgtccctgtggcctcttgggggtacatctcccggggctgggtcagaaggcctgggtggttggcctcaggctgtcacacacctagggagatgctcccgtttctgggaaccttggccccgactcctgcaaacttcggtaaatgtgtaactcgaccctgcaccggctcactctgttcagcagtgaaactctgcatcgatcactaagacttcctggaagaggtcccagcgtgagtgtcgcttctggcatctgtccttctggccagcctgtggtctggccaagtgatgtaaccctcctctccagcctgtgcacaggcagcctgggaacagctccatccccacccctcagctataaatagggcatcgtgacccggccgggggaagaagctgccgttgttctgggtactacagcagaagggtatgcggaagcgagcaccccagtctgagatggctcctgccggtgtgagcctgagggccaccatcctctgcctcctggcctgggctggcctggctgcaggtgaccgggtgtacatacaccccttccacctcgtcatccacaatgagagtacctgtgagcagctggcaaaggccaatgccgggaagcccaaagaccccaccttcatacctgctccaattcaggccaagacatcccctgtggatgaaaaggccctacaggaccagctggtgctagtcgctgcaaaacttgacaccgaagacaagttgagggccgcaatggtcgggatgctggccaacttcttgggcttccgtatatatggcatgcacagtgagctatggggcgtggtccatggggccaccgtcctctccccaacggctgtctttggcaccctggcctctctctatctgggagccttggaccacacagctgacaggctacaggcaatcctgggtgttccttggaaggacaagaactgcacctcccggctggatgcgcacaaggtcctgtctgccctgcaggctgtacagggcctgctagtggcccagggcagggctgatagccaggcccagctgctgctgtccacggtggtgggcgtgttcacagccccaggcctgcacctgaagcagccgtttgtgcagggcctggctctctatacccctgtggtcctcccacgctctctggacttcacagaactggatgttgctgctgagaagattgacaggttcatgcaggctgtgacaggatggaagactggctgctccctgatgggagccagtgtggacagcaccctggctttcaacacctacgtccacttccaagggaagatgaagggcttctccctgctggccgagccccaggagttctgggtggacaacagcacctcagtgtctgttcccatgctctctggcatgggcaccttccagcactggagtgacatccaggacaacttctcggtgactcaagtgcccttcactgagagcgcctgcctgctgctgatccagcctcactatgcctctgacctggacaaggtggagggtctcactttccagcaaaactccctcaactggatgaagaaactatctccccggaccatccacctgaccatgccccaactggtgctgcaaggatcttatgacctgcaggacctgctcgcccaggctgagctgcccgccattctgcacaccgagctgaacctgcaaaaattgagcaatgaccgcatcagggtgggggaggtgctgaacagcattttttttgagcttgaagcggatgagagagagcccacagagtctacccaacagcttaacaagcctgaggtcttggaggtgaccctgaaccgcccattcctgtttgctgtgtatgatcaaagcgccactgccctgcacttcctgggccgcgtggccaacccgctgagcacagcatgaggccagggccccagaacacagtgcctggcaaggcctctgcccctggcctttgaggcaaaggccagcagcagataacaaccccggacaaatcagcgatgtgtcacccccagtctcccaccttttcttctaatgagtcgactttgagctggaaagcagccgtttctccttggtctaagtgtgctgcatggagtgagcagtagaagcctgcagcggcacaaatgcacctcccagtttgctgggtttattttagagaatgggggtggggaggcaagaaccagtgtttagcgcgggactactgttccaaaaagaattccaaccgaccagcttgtttgtgaaacaaaaaagtgttcccttttcaagttgagaacaaaaattgggttttaaaattaaagtatacatttttgcattgccttcggtttgtatttagtgtcttgaatgtaagaacatgacctccgtgtagtgtctgtaataccttagttttttccacagatgcttgtgatttttgaacaatacgtgaaagatgcaagcacctgaatttctgtttgaatgcggaaccatagctggttatttctcccttgtgttagtaataaacgtcttgccacaataagcctccaaaaaaaa

SEQ ID NO: 2 - DNA, 18000 bp, Homo sapiens
cagagcaagaccccaactctaaaacaacacacaaaaatacagccatttctcctgggtgaaatgggggagctcagactattttgttttatttgtcaggagtctaaagcccatgtgagccaacttaagaaaattctgtttgtatttgagtgttctttattggaaagaaatggacttttccctaatgagcccattttacaaatcgagagctccaaatgcccggttccagcccccatgatatagatgggcagcaatgaggaccagaaatgctgggaagtgtccttgtcatgcaaggaaaacttggaacttcaaggatccatcatgggatgcaggacagtaggctccacccctcttcctgctttccagtaaatgatgttcagggctcacatgcctcttccaaggcatgatgtggggttgcagttctgatcccagcagagaacaaggctcctgtgaaacaattagttttggctcagaggcaaaaaatggaaaccccattcctgtatttacccttcattctttccttacctcatacagctggttccaggtttgattgcatcatatacataaataaataatctgctttcctggtttggtttagttttgctggagagaggagtttatgtgttcatcccatgactagctgggtggtcaagagattggaaagtaggagttctagtttagaccaagtctcatctcagaaaccacagagtagaactgatcccaaacgtcatcatccctgtagggaaaagaaagagagatcagactgttactgtgtctatatagaaagggaagacataagagactccattttgaaaaagagctatactttaaacaattgctttgctgagatgttgttaatttgtagctttgccccagccactttgacccaacctggagctcacaaaaacatgtgttgtataaaatcaaggtttaagggatctagggctgtgtcaaagtggctggggcaaagctacaaattaacaacatctcagcaaagcaattgtttaaagtacagctctttttcaaaatggagtctcttatgtcttccctttctatatagacacagtaacagtctgatctctcttttttttccctacatatcccaatagcacctgcctgactaatacatcatgctctgctgactccatatgtggctggtttcctggatccgattctgactgatggtatctgttctcacgctgctaataaagacataccagagactgggtaatttataaagaaaaagaggtttaatggacttatgtgttccacgtggctggggaggcctcacaatcatggtggaaggtgaaggaggagcaaaagcacatcttacatggtggctggcaaaagagagaaagcatgttcaggggaactcccctttataaaaccatcagatctcatgagacttatgcactatcacaagaacagcatcagaaagatccaccctcatgattcaattacctcccactgggtccctcccatgacacatgggaattatgggagctacaattggagatttgggtggggacacagccaaaccatatcagatggcttatttggtttctatgtagaacctctgcttttcattcaacagtcttcatttagccacagataagctctgtccctaacttccactgatggaatgtacacataagaaacttccactgatggaatgaacacagaaggtgcctactgggaagaaaactggcctgaatctgagctgggtcaaatgtctgcagtcagtttgaatggctgctccttatgggaataatttacattctcaataaaattctctagcaattttctgattgattttaatgagctttaaagccttacgtagaagatcccccagctgatagtcagccttgggcatggattaagggcttttaaccaatcttgcaacaagtttaagcagatattctttattgggtccaatctaaccaaaattattttcttatgttctccccagtaacgtgtcattattaagagaagtttggcttgcttagaggccaaatttagagggtcctgaaattttattttcttttacaccactttccagcatgttacctgatcagttgtttattatctttgctgttgaatggagtgatcattccaagggcccgaggcaggaggcccaggcacagtggaaactctcccaaagaccaggatctttgttttgttccctgacatatgctgagcaccaggaatagtgagtgaatgaaacaaattgtgaggctttaaagagccgaaatatttaaacactgggcacaaggttgttgcttaatcagtgctagatccttacctcccccttgtgtccaggtggacttgttactgcagttaaaccacttgctgatcctcaaacaactagttagtggcacagccaggcctaggaccccagtctctactgttccaactaacccattcgcaggcaggagcactttgaatggtctcttattttaaaaaaattaaattaaaattgtctatttatttagagacagagtcttactctgtagcccaggctcgagtgcagtggtgcaatcatagctcactgtaacctccatctcctggcctcaaaaagtgtttgaattacagatgcgaggcactgtacctggcccgaatgttctgttcagacaaagccacctctaagtcgctgtggggccccagacaagtgatttttgaggagtccctatctataggaacaaagtaattaaaaaaatgtatttcagaatttacaggcccatgtgagatatgatttttttaaatgaagatttagagtaatgggtaaaaaagaggtatttgtgtgtttgttgattgttcagtcagtgaatgtacagcttctgcctcatatccaggcaccatctcttcctgctctttgttgttaaatgttccattcctgggtaatttcatgtctgccatcgtggatatgccgtggctccttgaacctgcttgtgttgaagcaggatcttccttcctgtcccttcagtgccctaataccatgtatttaaggctggacacatcaccactcccaacctgcctcacccactgcgtcacttgtgatcactggcttctggcgactctcaccaaggtctctgtcatgccctgttataatgactacaaaagcaagtcttacctataggaaaataagaattataacccttttactggtcatgtgaaacttaccatttgcaatttgtacagcataaacacagaacagcacatctttcaatgcctgcatcctgaaggcattttgtttgtgtctttcaatctggctgtgctattgttggtgtttaacagtctccccagctacactggaaacttccagaaggcacttttcacttgcttgtgtgttttccccagtgtctattagaggcctttgcacagggtaggctctttggagcagctgaaggtcacacatcccatgagcgggcagcagggtcagaagtggcccccgtgttgcctaagcaagactctcccctgccctctgccctctgcacctccggcctgcatgtccctgtggcctcttgggggtacatctcccggggctgggtcagaaggcctgggtggttggcctcaggctgtcacacacctagggagatgctcccgtttctgggaaccttggccccgactcctgcaaacttcggtaaatgtgtaactcgaccctgcaccggctcactctgttcagcagtgaaactctgcatcgatcactaagacttcctggaagaggtcccagcgtgagtgtcgcttctggcatctgtccttctggccagcctgtggtctggccaagtgatgtaaccctcctctccagcctgtgcacaggcagcctgggaacagctccatccccacccctcagctataaatagggcatcgtgacccggccgggggaagaagctgccgttgttctgggtactacagcagaaggtaagccgggggccccctcagctccttctcggtcttgtctctctcagatgtaactgagctgtgggctaggaggaaaaggccgggaggaggcacggtgatgactgaaaaacctctcccctctcataagaccagtcatccggacgcgggctttcccccactcggtgcccacctggggtcttacaggaggagctgctcctcctcagcaataggacaagatggtcaggtcttcctgcttccgctgagaaaagttagggtcctcaggaacggagcagactggtacaggaacagagtcatcatggccaagagtccaccgggtcctcttgccatcaggaggaatagcagggcttgtgcaggaattggggctggagggaagggccgggctcggtcagtctccagctgggatccccagagtggtcaccctacccctccctcgagacagactgcctgactgtgtgtcatcaggctggtcaccatctccctgaacctcgatttgctcacctataaaatggaactaataacgatgcctgggctccctgtctcaggggctctggtatagctgaagagaactaatataacatgaaagtgctttctaagctttgggataagctaaaaggcagattccaattttattcgagggcagcgtagattggtgcttcagctcgtggatgacagagtcagggggcctggttctgagtcctagttctgtctcttcccagctgtgtgacgttgaacaagtcactggacctctctgttcctctgcaaaacagcatgaaccaattcattaactacttctccaggatgcagtaggtcccagggactatcctaggaatgtgggctgtattagtaaacacaacagcgggaaccctgttccggggctcacattcacatcagagcaaacagacaaagacgctggacagaataagtgcataactacatggtacagagggttataaggagggaaaaggggagctggatgagagagttgagagtgcccggtgtggtggggaaagctgcagggtgaaatactgcatcagggaaacctcagggaaggtgaggactatggtgaggtcagaggggttgatatgagaacagtgccctgcaaatggcaggcaccacaggagcatgagccgtcatcttcacctttagcattcagcccgggagaagtagggagacatagaaggggcaggtgctggccaagaggcaggggcaggagaggagaaggcggaggggcactcagggcgagggtgtcaggcccgccaccccagagcaccattactcccaggacgcggctgcgtgcagacctggaaccagcctagggagcagccgcagatcacaactgagaacaaacgacagtctctgcctcaaaaatggcccatggaattgcgtctctggagacgctgcctgagcaggagcagcacagtgagcgggctgcatcgaccagcgccatccaaaccccgaacagttggcgcttgtcaggcaggacttcccagcagtcggttcccacaggtttcccctgttgacctgatttgatgtgactgtctagattaggtgtgaactggtggcttaggcttctctgcacagaaaggcctgcaagcagcagagagagttttctgttccatttttccatgtcatgtggctcttcctgagaacagcggatggagtcaaatgcatggggagtggggtgagatggtagctgaggtcagaatttggcatttgaatgactgaagcagaacaaaacacaccaggtacttcagcagctgcaccgtgttgagggcaggtgctggttacgggtctgggtgagggaagccagctgccaatgtaagaagaatgactgggtatgcttagatgaagcagaaaaatctaggcatcaaggtggccttgagtcagtgatgacacgctacagctccaaggaagcctggcctagccctggggggacagaaaaggccaagaagtgacgatattgcagtacacccccctccacaagaaatgagtgagatgtggtacaaaatgttagaattgaatgaatcaatagaataaacgttcatcccttcaatcaagaagagtcagatgaaatgaattagcagggccagcccaagaacctcttctgggggtctcagggtagctttcatttgtagcagctgaggctgaagcccagctgcaaggcctttgagagaacgtggtgctggacccgtgtctagggcaggggttctaaaccctgcttacatatcagagtcacctgagaattttctatttttttttttttttttttatacgtggtcccagcacagactaaggaatccaactatcattgggcaagccatgctaggtatgcatgcctttggggctctgcaggggatagcgctatgcagggatggttgagagctggttttggggttgagacacgtgggaaatacttggactttgggctgagcctgtggtgctcaatcccggctgcatgttgggaccacagggagatgacaaaaccatccccagccctcaccctagggccctcgaatgagcatctcaggggtctaggaggcctccacaaagacctactgattggcacacacttgtttctctaggaagagaacttacagctgcaggcaggagcatgtcttaatctgcttgggctgccataagtaccacagactgggagggtttaacaacagaaatgtgttatctcacagttctggaagctagaagcctgggagccagccatcagcagagttggtttcctctgggtcctctatccttggcttgtagatggccgtcttctctctgtgtccccacatggtcttccctctgtgtccccacatggtcttccctctgtgtgtgtccatgtcctcatctcctcttctcataaggacacaggtcatattagatcagggctcaccctcatggcctcattttaacttaatcatctctttaaagatcctgtctccaaataatggtcacattctgaggtcctggggttgaggacttcaacacgggcattatggccgttgggggaggtaggacataattcagctgatattggtgcattttgcacttggatcatgtagatattttccatggagctttgaatccatttcttcttttttttgtagacatgaatggatttattctgggctaaatggtgacagggaatattgagacaatgaaagatctggttagatggcacttaaaggtcagttaataaccacctttcaccctttgcaaaatgatatttcagggtatgcggaagcgagcaccccagtctgagatggctcctgccggtgtgagcctgagggccaccatcctctgcctcctggcctgggctggcctggctgcaggtgaccgggtgtacatacaccccttccacctcgtcatccacaatgagagtacctgtgagcagctggcaaaggccaatgccgggaagcccaaagaccccaccttcatacctgctccaattcaggccaagacatcccctgtggatgaaaaggccctacaggaccagctggtgctagtcgctgcaaaacttgacaccgaagacaagttgagggccgcaatggtcgggatgctggccaacttcttgggcttccgtatatatggcatgcacagtgagctatggggcgtggtccatggggccaccgtcctctccccaacggctgtctttggcaccctggcctctctctatctgggagccttggaccacacagctgacaggctacaggcaatcctgggtgttccttggaaggacaagaactgcacctcccggctggatgcgcacaaggtcctgtctgccctgcaggctgtacagggcctgctagtggcccagggcagggctgatagccaggcccagctgctgctgtccacggtggtgggcgtgttcacagccccaggcctgcacctgaagcagccgtttgtgcagggcctggctctctatacccctgtggtcctcccacgctctctggacttcacagaactggatgttgctgctgagaagattgacaggttcatgcaggctgtgacaggatggaagactggctgctccctgatgggagccagtgtggacagcaccctggctttcaacacctacgtccacttccaaggtaaggcaaacctctctgctggctctggccctaggacttagtatccaatgtgtagctgagatcagccagtcaggccttggagatgggcagggggcagccctgcggacatacctggtgaccacccttgagaagtggggaagtggctgctccgctgggtccctggatgggccgtccacctcctggacctgctgccctactatgtgcacgactatacaacatcctttttcttacatcatttaatccccttatgatgtggtgaagaggtatttgtgcctttgtttaccagtgaagaaatagagactcggagaaacaaagtgccttgctcaagatggcacagccaccagtgggggtcctgggattgaaacccacatctcctggccccacagcccagttctacactcagaagggtcaggttcatatctcttgagaaggtcaggaactggggtccctggcccatgcagaaataagcaattggcttgcttaaatccctttcatgttaggaggggcattactgaaaaccctctactacaaagattgttgatttttttttttttttttattgagacagggtcttgttctgtcacccaggctgcagtgtagtggtgccatcattgctcactgtagccttgaactcctggcctcaagcgatcctcccacctctgccttccaaagtgttgggattaaaggtgtgagccactgcacccagccacagattgcttaaagcattcatttaacaaatacttgttgaggatttgctacttgtaagactttaagcctggcatctcagaggaggccagaggagggctgtataggccctgcctccaggcttttaaaggtcaatgggcaaatgcctaggatttggagctgcagggaaacgtgctccacaaggtaactcagggaagcctcggggctctcagaggacagaggtcactggggagcggagagcaggccttgcctggcagtgagggcaacagggctggtgaagctaggagcaagcatgatgagcccagcctgcagagtttggggcaaggaacgaggatggggcggttggcttggcatgagtgttgaaccagaaaatgggcctggggagggcagagctggagacactttgaacgccatgcttggtaggtgtgggaatggggacgcgttctgttcagaggtcatcccggaagcctgccgtgtgcagactggaggcagggaggattgtttgaaggttacgcaagagtccaggcacacagtcacgggaacacgtgctcagggagcagctcggcaaatccatgggtggggtggggctgaggggtgtgtctaagagacactgaggaggctctgtcaagatgttaacctcgtgagggacagagagccaggcgggaggtgaaagacaagactgtggagaaagaggttcagtggcgcatagtgatttttcttaccacaacaacctccttgaggtctttcccttcgggttcagggagaggtgatagatggggggattgctcagccctggcactgactggtcacaggggcagaggccagcccgagggttgcccggttgagggtggcagcacactgtgcagggcagagcagggacacatggacttagcctgctgtccctaggagaagtgctgggaggagcgctcactgagaaggagggtcctgcagaaggcaaaggcaagaaagccagtggcatctgaaatgggtctcccttcgaaagagagcacatccacctgacccagaccgcagagccaggccaggaggaagaggaggaagaataaaaaagccaaccacatcgggactcaaaggaagcccaggatcctcgccggcctccaccgcatgctgccctgaccctgccccacttcctaactttgctggcctcagtttccgtcaaaggaggcagccacttcctgcccacatggtctgtccagtgaggagatcgggggctgtctcgggacctctaggtttccctttagcaatgatgttctatttacatgacctcagcaggcagctagatgtgtcccactagagaggacctgaggatctggggcctgatgggctccagggtaccgtctgcccagtgcttgctgtgctcctgagcatggggcgctggccctggtggtttccatgacaccaggtcctgacttgacctcgacagatttacctagcctccggatgagaatggtgagctgtgcatgtcagacgagcagagggaagacggcagccactctcatgtcaaatcccagcgtcttttgggaggcagcttcccttttttagtttagtttgttggaagaaaagaattgtccctttcccccctctaaactaaaagccttgccagcccaggtgggcagcaccgaggtccctgcagggaacgtgcaaggggaaccctgcagtttcccgctcacatgcccttccgagactgagtgctccgaggactgaggacgagaaatatgccaggtctgccactgccttcttacgagacccggacccaggggaggcacagccatgcccagctcctgcctgccagttctgtcctcccagctgccctactttcatgctgggacctccaattcagtacaaagggagacctcactgtttctgaaccatctctactcagactcccaagtgccacgtgcccaggggactgttctgtgacaaacttatacacaacttcaccctattctcctaagaacaaccgcagaataggcctttcaggatgagtgggaggacagccgagggcagggatgtgctagtgtaaggtcgaggcagagggtgggctgctgtcatggaaagaccccaggtaactgcgtcacacacaaatttgtgtccttctcccacaacgggctctcccgagttctctgtcatctgcacggccctgtgagcaggaggggaaacagagggctcacccctgcccccaaggcccagtgtgcaaatccattcatcacaacgaggttgtgtgagtctccccagtagcaagggctgctgaggaatggagccctcgtttccggggcctgcgtggcccactctgtattctatgactgtgatgggggagggtgggggccacaggacagctggtgggctctgccatggctggggctagacatggattaaaaagtgagtatgagcaggggcctctaggagtggtgggatagtgcggtggtggccacatgtcattctacgtgcgtccaaacctacagaatgtaaaacaccaggagggagactcaaagaaaactatcaactttgagtgctgaggacgtgtcagtgtaggttcgtcagttgcaacaaatgggccacgctggtgtgagatgttgatcacgggggaggctgtgtagtgggggacaagagttatatgggaactttctgtactttctgctcgattttgctgtgaacctaaagtcactctaaaaaataacatctcttaaattttttaaaaagtgagtgtgtcaaaccacagcctttgggtcaggacagttctaggtttgagttgacctggcaggtaccagtggcttatgtcccttaaggtgacagatgcaaaacccccggtttggtgcctggcatgttgtgtgtcttgcaggtggcggttagggctgcctcagtgaactcaaatggctgcattttacaggagaaatatttgagccacacttgcggtcctgtggccaggagaatgcagagtggcctggggggggccaaggaaggaggctgaggcagggcgaggggcaggatctgggcctttggtgtctgccagccctcattcctgcccctgtcttgggtgactcttccctccctgtctcctgtctggatttcagggaagatgaagggcttctccctgctggccgagccccaggagttctgggtggacaacagcacctcagtgtctgttcccatgctctctggcatgggcaccttccagcactggagtgacatccaggacaacttctcggtgactcaagtgcccttcactgagagcgcctgcctgctgctgatccagcctcactatgcctctgacctggacaaggtggagggtctcactttccagcaaaactccctcaactggatgaagaaactatctccccggtaggagcctcccggtctcccctggaatgtgggagccacactgtcctgcccaggctgggggcggggtggggagtagacacacctgagctgagccttgggtgcagagcagggcagggccgcggtggcacggggctgggcaggcggcctgtgtgtctgtctaccagtcctctatccagccagcacccagctctccagttagtgtctgtctttcaagtgcaggcaaggtaaaggaggagaggaagaatgctttttctacacttacacttgcctggtagttttggagggggagaaaacattgcaatccgccctctgagagaggaccattttggtcccacacctgacacacagcacacctgtgacatccaagagcttcttggaactgacttgccaggagggttcggacttcgcgtgagcgggggtggggccttctcagggagcgtcccttgactccagaacgcccttgctggcggctggcggctgggtggggataggtgttgttagctcctctttcctgctgcaattcctttccacagagccctggactcaaactacacatcaccccagatcatcgaggcctggaaatctgctcccagaggcaggcattgagtgacacgatggcttgacatcaactctgggtgttttttatgttttaaaaattgtgatggtaaaatatacgtaacaaaatttgccatcgtaaccattttcgagtgcacagttcagtggtactaggcccattcacactgttgtgcagccatcacccccgtccatctccatttatcttctcaacttcccaaactgaagctctgtcctgctgaaacactaactctccatttccccttccccttggccccggcaaccaccacgatgtcctcgaggttcacccatgttgtagcacatgtcagaatgtccttccttttgaaggctgaataatattccattgcatgtggttaccaccttttgtgtatccactcatccatcgatggacacgtgggttgcttccacctttgagctgctgtgaatagtgcagtgtaccctgtaaacatgggtgtactgtcagctcttataagtgcttgatacatcactggaaatgtccatgggctctgaaggatgccaaaagatggaagaggctctatacgaagatcaatcgagttgacatagcaacgtgtccagcacgaggttgacactgtaccctcctgcctctctccttttcatgggtgtcatgtcatcaagaacactgctgtggcagtagtaagacacagtgcattatttcagagaatagcatttaaaaattacccaagtaacacaccttcaatgcagccaacctaaaaacagaatgcaccaaaggacaaccattcctaggtcctcatcggtaaatcttctatgtccctcacatagtattgcaaatgacatgaaggatttttattgtaggttttgctgaaattttccccaagggggaggatgacttagttgggtgatggggggagcaaacatccctgtcgtcagggttgggtgcaaggagcataagcctgcctggcctctgggagagccctcactgtgtggcctggagccttcctaactgtgcatcatctccccaggaccatccacctgaccatgccccaactggtgctgcaaggatcttatgacctgcaggacctgctcgcccaggctgagctgcccgccattctgcacaccgagctgaacctgcaaaaattgagcaatgaccgcatcagggtgggggaggtatgtgtgagcctgtgtctgtgcctgacctgggttccaagtgtgcacagggtgggaggcatggatgtaagggacacagaggaggctatgggtggggccagcagggcaagagggagcggagagtagggccaaaggtgggagagaagtagccagagcattctggggccttccaggtgcagagcagcaaatccctccccatccctgctgtgcctcctcctgctaggtgtgtgttccatggtcctgcttggccttgccttgcctcagggtcctccagggttcctatagtggagttgaaaccgggatgaagacagcaagcacccctggacctggtgccctgggcccagccccttcttcagggaaatgctgagcagcagacagaatgtccccctgccatgtggcaccatgcacatctgcagctaccaaggatgtgccttgatgttctgggccctgtgctcagtgctggggagaaagtgggagttcttacgggggccagcgggaagagccctctgtgctaagttagctaagccctggcactggtgggccatggccaagggagccaggaattctgcctgggacatcagggcagaatgtgaagatgggaggatgtaaggggtgtgttagggaggagccggcatgtgagtttggccattgtggccaattaacggtcatctacacacagacacacccttgcctacactgaggggcaggcatacactgtgcatcctcctggcaggctggaaaatgtccccctccaggacagtgcacagcacagaggtcctgagcccaccccggccctctagccctcagcaccctgggtcacccagtgcgccctcagaatgatcctgatgtctgctgctttgcaggtgctgaacagcattttttttgagcttgaagcggatgagagagagcccacagagtctacccaacagcttaacaagcctgaggtcttggaggtgaccctgaaccgcccattcctgtttgctgtgtatgatcaaagcgccactgccctgcacttcctgggccgcgtggccaacccgctgagcacagcatgaggccagggccccagaacacagtgcctggcaaggcctctgcccctggcctttgaggcaaaggccagcagcagataacaaccccggacaaatcagcgatgtgtcacccccagtctcccaccttttcttctaatgagtcgactttgagctggaaagcagccgtttctccttggtctaagtgtgctgcatggagtgagcagtagaagcctgcagcggcacaaatgcacctcccagtttgctgggtttattttagagaatgggggtggggaggcaagaaccagtgtttagcgcgggactactgttccaaaaagaattccaaccgaccagcttgtttgtgaaacaaaaaagtgttcccttttcaagttgagaacaaaaattgggttttaaaattaaagtatacatttttgcattgccttcggtttgtatttagtgtcttgaatgtaagaacatgacctccgtgtagtgtctgtaataccttagttttttccacagatgcttgtgatttttgaacaatacgtgaaagatgcaagcacctgaatttctgtttgaatgcggaaccatagctggttatttctcccttgtgttagtaataaacgtcttgccacaataagcctccaaaaattttatctttcatttagcagccaaacagatgtatacaattcagcagatagactgtgcaaacgaaagtgctttcctggactttggatggaatttccatgggaggtctgagccagtacttagcagtcctttgaagttttaggtgatgcttttctctggacacttccattggtaagcagtggtggccatctgtgtgatggacagggggcgggaagagggtgacagggaaggccccataccccatgtggcacctgggaaaggaaccaggcagatgggacttcttccgtcctggtgacacagggccagactgctgctggtattgtgccccgggagtggaaggtagagaaataaatcttcacaaataaatatttgcaattttcccccatctgttgagtgcctctgcctgctcctcctcgatgggattaggcccacagttcggaatcttggggagagccaaggaagcggtaggcacccagtaggcccacggccgtcggctgatagcaatggtgatgctgtcctacctacttgtgtaaggcattcgatcttcctcccttccatacatattgaaataaataagccgcgcaatgtgttagctattgatcagaactaaagtgaagtcagccacggggattacaaatctcggcttctcccctcatgttcctgagagtcttcccctggttttgaacacatctccctagctcgatgtcaaggtgagggattctgtcggcaacagcagtgcccttagttgcttcgtcgtaactccccgtcaccggttttattcagttaccttccagtcccactctcagagcttcctggcttgttctgctctcaaagcgggtagagctggcacacatggactctccgaaacggctgcaagatgccaagtttctcggaagaactggaagcacagagaccagaagtgccttaaggtctcgctattcagtgtggcgcttagaccggcagtggcggcagctgccctgggagcttgttagaatgtggcttctcacgcccctcctggacctacagagtcagaatctgcagttttacaggaggtccaggcttggaagttgctcgtagagacctgagacagcgcagccacgtgctggaaacaaagcatttaagtttgtgactttattttaaaaggcagcaggcagtcgacaaaccaatttcttctacttagaggcggcttcggcttctggaagtcgctaggagtataaagttgccaaccagcgctgttctcccgctgttttctgtgcacttataaatgggaagttaggtcaggatagatctctcagctattacaaggatacaaaatacgaacattctacaagttacttaacacacacacacacacacacacacacacacacacacacaaaattaattccacaggtcagtttctctgaaacattttttcactaaattctaagtcttcctggagttgcaagtgcctatctcctagacaaggcaattactcaccaactaaaatcactgtcaatctgagatttcggctgggcatgagaccatggtcaggggatgctttgaacagcctctgaggaaattagtgagtttgaaaaatggaaagatttttattactcacttggcagtaaaacctgatggggacagacgtcaggctgtttaagatcctcagaagaaaaagttgatagtgtgaatattcctaaatttgccacacgaagatgtacatgtgattataaggtgctgttgcagaagcccctgggggtgttatgggatatacactatatgggccactttaccttcctaaaatctgaaaaacttcaactactgaaacatggactgaaggttttgaatagtggatggtgaatttgaataccatcccgtgtgatttttttttctagcagactttagttttttagagcagttttaagcccacaccaaaactgagaggaagatacagcaatttctcatataccccctactaccttccagtctcccccattattgacatcccccacccagagtggtccatttcttacaacccacgaacctacattgacacatcattattactcaacgtccatagtttacattagggttggctcttggtgttgtacattctatgggtttagacaattttcaggagtttcactgacctgaaaatcctctgtgtccctcctattcacccctccttccctcctaaccactggtaaccaccgatcctattcccatcttctccatagttttgcctttcccacccaggatgtcatatagtggaatcattcagtatgtggcctttccagattagcctctttcacttagtaatgtgcatttaagtttcctccatgtcttttcatgatcgctcatttcttttttattgctaaatactatgccactgtctggatgtgtcacagtttatttattcacctactgaaggacatcttgcttgtttccaagttgtggcaattgcgaattaagctgctacagacacccatgtgtgggtttttgtgtggacatgtttaccccacacaatttttaaagttgctcaa

SEQ ID NO: 3 - DNA, 19 bp, Artificial sequence
  Primer
ccctgatgggagccagtgt

SEQ ID NO: 4 - DNA, 19 bp, Artificial sequence
  Primer
agcagggagaagcccttca

SEQ ID NO: 5 - DNA, 27 bp, Artificial sequence
  Probe
ccctggctttcaacacctacgtccact

SEQ ID NO: 6 - DNA, 20 bp, Artificial sequence
  Primer
ggacaaggtggagggtctca

SEQ ID NO: 7 - DNA, 21 bp, Artificial sequence
  Primer
agatccttgcagcaccagttg

SEQ ID NO: 8 - DNA, 29 bp, Artificial sequence
  Probe
atgaagaaactatctccccggaccatcca

SEQ ID NO: 9 - DNA, 19 bp, Artificial sequence
  Primer
gaaggtgaaggtcggagtc

SEQ ID NO: 10 - DNA, 20 bp, Artificial sequence
  Primer
gaagatggtgatgggatttc

SEQ ID NO: 11 - DNA, 20 bp, Artificial sequence
  Probe
caagcttcccgttctcagcc

SEQ ID NO: 12 - DNA, 16 bp, Artificial sequence
  Synthetic oligonucleotide
cgctgatttgtccggg

SEQ ID NO: 13 - DNA, 16 bp, Artificial sequence
  Synthetic oligonucleotide
tcggttggaattcttt

SEQ ID NO: 14 - DNA, 16 bp, Artificial sequence
  Synthetic oligonucleotide
  misc_feature (5)..(5): bases at these positions are RNA
tcggutggaattcttt

SEQ ID NO: 15 - DNA, 16 bp, Artificial sequence
  Synthetic oligonucleotide
gtcggttggaattctt

SEQ ID NO: 16 - DNA, 16 bp, Artificial sequence
  Synthetic oligonucleotide
  misc_feature (6)..(6): bases at these positions are RNA
ctcatugtggatgacg

SEQ ID NO: 17 - DNA, 16 bp, Artificial sequence
  Synthetic oligonucleotide
ctcattgtggatgacg

SEQ ID NO: 18 - DNA, 16 bp, Artificial sequence
  Synthetic oligonucleotide
  misc_feature (6)..(6): bases at these positions are RNA
tgaatuggagcaggta

SEQ ID NO: 19 - DNA, 16 bp, Artificial sequence
  Synthetic oligonucleotide
tgaattggagcaggta

SEQ ID NO: 20 - DNA, 16 bp, Artificial sequence
  Synthetic oligonucleotide
cggtgtcaagttttgc

SEQ ID NO: 21 - DNA, 16 bp, Artificial sequence
  Synthetic oligonucleotide
gttgggtagactctgt

SEQ ID NO: 22 - DNA, 16 bp, Artificial sequence
  Synthetic oligonucleotide
gttggaattctttttg

SEQ ID NO: 23 - DNA, 16 bp, Artificial sequence
  Synthetic oligonucleotide
gttaagctgttgggta

SEQ ID NO: 24 - DNA, 16 bp, Artificial sequence
  Synthetic oligonucleotide
  misc_feature (5)..(5): bases at these positions are RNA
tgaautggagcaggta

SEQ ID NO: 25 - DNA, 16 bp, Artificial sequence
  Synthetic oligonucleotide
ttgcaggttcagctcg

SEQ ID NO: 26 - DNA, 16 bp, Artificial sequence
  Synthetic oligonucleotide
ggtagactctgtgggc

SEQ ID NO: 27 - DNA, 16 bp, Artificial sequence
  Synthetic oligonucleotide
gttggaattctttttg

SEQ ID NO: 28 - DNA, 20 bp, Artificial sequence
  Synthetic oligonucleotide
cacaaacaagctggtcggtt